European Patent Application EP 4 755 911 A2, published June 10, 2026. Title: ANTIBODY PAIR FOR BINDING TO MATURE PROLACTIN. Applicant: SHENZHEN MINDRAY BIO-MEDICAL ELECTRONICS CO., LTD. The sequence listing filed with the application follows.

SEQUENCE LISTING (59 sequences)

SEQ ID NO: 1 - protein, 199 aa, Homo sapiens
LPICPGGAARCQVTLRDLFDRAVVLSHYIHNLSSEMFSEFDKRYTHGRGFITKAINSCHTSSLATPEDKEQAQQMNQKDFLSLIVSILRSWNEPLYHLVTEVRGMQEAPEAILSKAVEIEEQTKRLLEGMELIVSQVHPETKENEIYPVWSGLPSLQMADEESRLSAYYNLLHCLRRDSHKIDNYLKLLKCRIIHNNNC

SEQ ID NO: 2 - protein, 13 aa, Homo sapiens
LPICPGGAARCQV

SEQ ID NO: 3 - protein, 17 aa, Homo sapiens
DNYLKLLKCRIIHNNNC

SEQ ID NO: 4 - protein, 447 aa, synthetic construct
EVMSAESGGGLVKPGGSLKFSCAASWFGFSGFIFSWYVVWRQTPMERLFWVAISGGDSHTRFNISRNNAKNLTLYLMQSSLRSNATAMYYCWRTRHSPYDHGDFGYVGQGATLTVSSAKTTAPSVYPLAPVCGDTTGSSVTLGCLVKGYFPEPVTLTWNSGSLSSGVHTFPAVLQSDLYTLSSSVTVTSSTWPSQSITCNVAHPASSTKVDKKIEPRGPTIKPCPPCKCPAPNLLGGPSVFIFPPKIKDVLMISLSPIVTCVVVDVSEDDPDVQISWFVNNVEVHTAQTQTHREDYNSTLRVVSALPIQHQDWMSGKEFKCKVNNKDLPAPIERTISKPKGSVRAPQVYVLPPPEEEMTKKQVTLTCMVTDFMPEDIYVEWTNNGKTELNYKNTEPVLDSDGSYFMYSKLRVEKKNWVERNSYSCSVVHEGLHNHHTTKSFSRTPGK

SEQ ID NO: 5 - protein, 117 aa, synthetic construct
EVMSAESGGGLVKPGGSLKFSCAASWFGFSGFIFSWYVVWRQTPMERLFWVAISGGDSHTRFNISRNNAKNLTLYLMQSSLRSNATAMYYCWRTRHSPYDHGDFGYVGQGATLTVSS

SEQ ID NO: 6 - protein, 8 aa, synthetic construct
GFIFSWYV

SEQ ID NO: 7 - protein, 8 aa, synthetic construct
ISGGDSHT

SEQ ID NO: 8 - protein, 13 aa, synthetic construct
TRHSPYDHGDFGY

SEQ ID NO: 9 - protein, 211 aa, synthetic construct
DAMVTQESALTTSPGETVTLTCQTLVHSLGNTYWVQEKPDHLFTGLIGKVSIAGVPDRFSGSGSGTDFTLKISRVEAEDLGVYFCSQTTHVPTFFGGGTKLEIKRADAAPTVSIFPPSSEQLTSGGASVVCFLNNFYPKDINVKWKIDGSERQNGVLNSWTDQDSKDSTYSMSSTLTLTKDEYERHNSYTCEATHKTSTSPIVKSFNRNEC

SEQ ID NO: 10 - protein, 104 aa, synthetic construct
DAMVTQESALTTSPGETVTLTCQTLVHSLGNTYWVQEKPDHLFTGLIGKVSIAGVPDRFSGSGSGTDFTLKISRVEAEDLGVYFCSQTTHVPTFFGGGTKLEIK

SEQ ID NO: 11 - protein, 11 aa, synthetic construct
QTLVHSLGNTY

SEQ ID NO: 12 - protein, 5 aa, synthetic construct
KVSIA

SEQ ID NO: 13 - protein, 9 aa, synthetic construct
SQTTHVPTF

SEQ ID NO: 14 - protein, 441 aa, synthetic construct
EVMLVESGGGLVRPGGSLKLSCAASGFTFSGASITSDYAWVRQTPEKRLEWVAISFGGGHTRFTISRDNAKNTLYLQMSSLKSDDTAMYYCARARHSPNDHGDTNFWGQGTTLAVSSAKTTPPSVYPLAPGSAAQTNSMVTLGCLVKGYFPEPVTVTWNSGSLSSGVHTFPAVLQSDLYTLSSSVTVPSSTWPSETVTCNVAHPASSTKVDKKIVPRDCGCKPCICTVPEVSSVFIFPPKPKDVLTITLTPKVTCVVVDISKDDPEVQFSWFVDDVEVHTAQTQPREEQFNSTFRSVSELPIMHQDWLNGKEFKCRVNSAAFPAPIEKTISKTKGRPKAPQVYTIPPPKEQMAKDKVSLTCMITDFFPEDITVEWQWNGQPAENYKNTQPIMDTDGSYFVYSKLNVQKSNWEAGNTFTCSVLHEGLHNHHTEKSLSHSPGK

SEQ ID NO: 15 - protein, 117 aa, synthetic construct
EVMLVESGGGLVRPGGSLKLSCAASGFTFSGASITSDYAWVRQTPEKRLEWVAISFGGGHTRFTISRDNAKNTLYLQMSSLKSDDTAMYYCARARHSPNDHGDTNFWGQGTTLAVSS

SEQ ID NO: 16 - protein, 9 aa, synthetic construct
GASITSDYA

SEQ ID NO: 17 - protein, 8 aa, synthetic construct
ISFGGGHT

SEQ ID NO: 18 - protein, 13 aa, synthetic construct
ARHSPNDHGDTNF

SEQ ID NO: 19 - protein, 208 aa, synthetic construct
DVVMTQTPLSLPVSLGDQSSISCQDISDNGWYLQKPVQSPKLLIYKTSGVGVPDCFSGSGSGTDFSLKISRVETEDLGVYFCQQGNTVPLTFGGGTKLEIKRADAAPTVSIFPPSSEQLTSGGASVVCFLNNFYPKDINVKWKIDGSERQNGVLNSWTDQDSKDSTYSMSSTLTLTKDEYERHNSYTCEATHKTSTSPIVKSFNRNEC

SEQ ID NO: 20 - protein, 101 aa, synthetic construct
DVVMTQTPLSLPVSLGDQSSISCQDISDNGWYLQKPVQSPKLLIYKTSGVGVPDCFSGSGSGTDFSLKISRVETEDLGVYFCQQGNTVPLTFGGGTKLEIK

SEQ ID NO: 21 - protein, 7 aa, synthetic construct
QDISDNG

SEQ ID NO: 22 - protein, 5 aa, synthetic construct
KTSGV

SEQ ID NO: 23 - protein, 9 aa, synthetic construct
QQGNTVPLT

SEQ ID NO: 24 - protein, 8 aa, synthetic construct
  VARIANT 5: note = X is S, T, A or G.
GFIFXWYV

SEQ ID NO: 25 - protein, 8 aa, synthetic construct
GFIFTWYV

SEQ ID NO: 26 - protein, 8 aa, synthetic construct
GFIFAWYV

SEQ ID NO: 27 - protein, 8 aa, synthetic construct
GFIFGWYV

SEQ ID NO: 28 - protein, 8 aa, synthetic construct
  VARIANT 5: note = X is D, E, Q or N
ISGGXSHT

SEQ ID NO: 29 - protein, 8 aa, synthetic construct
ISGGESHT

SEQ ID NO: 30 - protein, 8 aa, synthetic construct
ISGGQSHT

SEQ ID NO: 31 - protein, 8 aa, synthetic construct
ISGGNSHT

SEQ ID NO: 32 - protein, 117 aa, synthetic construct
EVMSAESGGGLVKPGGSLKFSCAASWFGFSGFIFSWYVVWRQTPMERLFWVAISGGESHTRFNISRNNAKNLTLYLMQSSLRSNATAMYYCWRTRHSPYDHGDFGYVGQGATLTVSS

SEQ ID NO: 33 - protein, 117 aa, synthetic construct
EVMSAESGGGLVKPGGSLKFSCAASWFGFSGFIFSWYVVWRQTPMERLFWVAISGGQSHTRFNISRNNAKNLTLYLMQSSLRSNATAMYYCWRTRHSPYDHGDFGYVGQGATLTVSS

SEQ ID NO: 34 - protein, 117 aa, synthetic construct
EVMSAESGGGLVKPGGSLKFSCAASWFGFSGFIFSWYVVWRQTPMERLFWVAISGGNSHTRFNISRNNAKNLTLYLMQSSLRSNATAMYYCWRTRHSPYDHGDFGYVGQGATLTVSS

SEQ ID NO: 35 - protein, 117 aa, synthetic construct
EVMSAESGGGLVKPGGSLKFSCAASWFGFSGFIFTWYVVWRQTPMERLFWVAISGGDSHTRFNISRNNAKNLTLYLMQSSLRSNATAMYYCWRTRHSPYDHGDFGYVGQGATLTVSS

SEQ ID NO: 36 - protein, 117 aa, synthetic construct
EVMSAESGGGLVKPGGSLKFSCAASWFGFSGFIFTWYVVWRQTPMERLFWVAISGGESHTRFNISRNNAKNLTLYLMQSSLRSNATAMYYCWRTRHSPYDHGDFGYVGQGATLTVSS

SEQ ID NO: 37 - protein, 117 aa, synthetic construct
EVMSAESGGGLVKPGGSLKFSCAASWFGFSGFIFTWYVVWRQTPMERLFWVAISGGQSHTRFNISRNNAKNLTLYLMQSSLRSNATAMYYCWRTRHSPYDHGDFGYVGQGATLTVSS

SEQ ID NO: 38 - protein, 117 aa, synthetic construct
EVMSAESGGGLVKPGGSLKFSCAASWFGFSGFIFTWYVVWRQTPMERLFWVAISGGNSHTRFNISRNNAKNLTLYLMQSSLRSNATAMYYCWRTRHSPYDHGDFGYVGQGATLTVSS

SEQ ID NO: 39 - protein, 117 aa, synthetic construct
EVMSAESGGGLVKPGGSLKFSCAASWFGFSGFIFAWYVVWRQTPMERLFWVAISGGDSHTRFNISRNNAKNLTLYLMQSSLRSNATAMYYCWRTRHSPYDHGDFGYVGQGATLTVSS

SEQ ID NO: 40 - protein, 117 aa, synthetic construct
EVMSAESGGGLVKPGGSLKFSCAASWFGFSGFIFAWYVVWRQTPMERLFWVAISGGESHTRFNISRNNAKNLTLYLMQSSLRSNATAMYYCWRTRHSPYDHGDFGYVGQGATLTVSS

SEQ ID NO: 41 - protein, 117 aa, synthetic construct
EVMSAESGGGLVKPGGSLKFSCAASWFGFSGFIFAWYVVWRQTPMERLFWVAISGGQSHTRFNISRNNAKNLTLYLMQSSLRSNATAMYYCWRTRHSPYDHGDFGYVGQGATLTVSS

SEQ ID NO: 42 - protein, 117 aa, synthetic construct
EVMSAESGGGLVKPGGSLKFSCAASWFGFSGFIFAWYVVWRQTPMERLFWVAISGGNSHTRFNISRNNAKNLTLYLMQSSLRSNATAMYYCWRTRHSPYDHGDFGYVGQGATLTVSS

SEQ ID NO: 43 - protein, 117 aa, synthetic construct
EVMSAESGGGLVKPGGSLKFSCAASWFGFSGFIFGWYVVWRQTPMERLFWVAISGGDSHTRFNISRNNAKNLTLYLMQSSLRSNATAMYYCWRTRHSPYDHGDFGYVGQGATLTVSS

SEQ ID NO: 44 - protein, 117 aa, synthetic construct
EVMSAESGGGLVKPGGSLKFSCAASWFGFSGFIFGWYVVWRQTPMERLFWVAISGGESHTRFNISRNNAKNLTLYLMQSSLRSNATAMYYCWRTRHSPYDHGDFGYVGQGATLTVSS

SEQ ID NO: 45 - protein, 117 aa, synthetic construct
EVMSAESGGGLVKPGGSLKFSCAASWFGFSGFIFGWYVVWRQTPMERLFWVAISGGQSHTRFNISRNNAKNLTLYLMQSSLRSNATAMYYCWRTRHSPYDHGDFGYVGQGATLTVSS

SEQ ID NO: 46 - protein, 117 aa, synthetic construct
EVMSAESGGGLVKPGGSLKFSCAASWFGFSGFIFGWYVVWRQTPMERLFWVAISGGNSHTRFNISRNNAKNLTLYLMQSSLRSNATAMYYCWRTRHSPYDHGDFGYVGQGATLTVSS

SEQ ID NO: 47 - protein, 7 aa, synthetic construct
  VARIANT 5: note = X is D or E.
QDISXNG

SEQ ID NO: 48 - protein, 7 aa, synthetic construct
QDISENG

SEQ ID NO: 49 - protein, 5 aa, synthetic construct
  VARIANT 4: note = X is G, A, S or T.
KTSXV

SEQ ID NO: 50 - protein, 5 aa, synthetic construct
KTSAV

SEQ ID NO: 51 - protein, 5 aa, synthetic construct
KTSSV

SEQ ID NO: 52 - protein, 5 aa, synthetic construct
KTSTV

SEQ ID NO: 53 - protein, 101 aa, synthetic construct
DVVMTQTPLSLPVSLGDQSSISCQDISDNGWYLQKPVQSPKLLIYKTSAVGVPDCFSGSGSGTDFSLKISRVETEDLGVYFCQQGNTVPLTFGGGTKLEIK

SEQ ID NO: 54 - protein, 101 aa, synthetic construct
DVVMTQTPLSLPVSLGDQSSISCQDISDNGWYLQKPVQSPKLLIYKTSSVGVPDCFSGSGSGTDFSLKISRVETEDLGVYFCQQGNTVPLTFGGGTKLEIK

SEQ ID NO: 55 - protein, 101 aa, synthetic construct
DVVMTQTPLSLPVSLGDQSSISCQDISDNGWYLQKPVQSPKLLIYKTSTVGVPDCFSGSGSGTDFSLKISRVETEDLGVYFCQQGNTVPLTFGGGTKLEIK

SEQ ID NO: 56 - protein, 101 aa, synthetic construct
DVVMTQTPLSLPVSLGDQSSISCQDISENGWYLQKPVQSPKLLIYKTSGVGVPDCFSGSGSGTDFSLKISRVETEDLGVYFCQQGNTVPLTFGGGTKLEIK

SEQ ID NO: 57 - protein, 101 aa, synthetic construct
DVVMTQTPLSLPVSLGDQSSISCQDISENGWYLQKPVQSPKLLIYKTSAVGVPDCFSGSGSGTDFSLKISRVETEDLGVYFCQQGNTVPLTFGGGTKLEIK

SEQ ID NO: 58 - protein, 101 aa, synthetic construct
DVVMTQTPLSLPVSLGDQSSISCQDISENGWYLQKPVQSPKLLIYKTSSVGVPDCFSGSGSGTDFSLKISRVETEDLGVYFCQQGNTVPLTFGGGTKLEIK

SEQ ID NO: 59 - protein, 101 aa, synthetic construct
DVVMTQTPLSLPVSLGDQSSISCQDISENGWYLQKPVQSPKLLIYKTSTVGVPDCFSGSGSGTDFSLKISRVETEDLGVYFCQQGNTVPLTFGGGTKLEIK